European Patent Application EP 4 502 602 A1, published February 5, 2025. Title: 免疫学的検出方法及び免疫学的検出キット. Applicant: 積水メディカル株式会社. Application WO. The sequence listing filed with the application follows.

SEQUENCE LISTING (7 sequences)

SEQ ID NO: 1 - protein, 10 aa, Homo sapiens
QEEGQVEGQD

SEQ ID NO: 2 - protein, 13 aa, Homo sapiens
PDGSESPTDQETT

SEQ ID NO: 3 - protein, 10 aa, Homo sapiens
QSLQEETVRK

SEQ ID NO: 4 - protein, 10 aa, Homo sapiens
  NON_STD 1: note = L-Pyroglutamic Acid
ESLQEETVRK

SEQ ID NO: 5 - protein, 11 aa, Homo sapiens
QEEGQVEGQDC

SEQ ID NO: 6 - protein, 14 aa, Homo sapiens
PDGSESPTDQETTC

SEQ ID NO: 7 - protein, 11 aa, Homo sapiens
  NON_STD 1: note = L-Pyroglutamic Acid
ESLQEETVRKC